European Patent Application EP 4 534 524 A1, published April 9, 2025. Title: Amino Acid Active Esther and Salts Thereof. Applicant: PeptiDream Inc. Application JP. The sequence listing filed with the application follows.

SEQUENCE LISTING (4 sequences)

SEQ ID NO: 1 - RNA, 45 nt, synthetic construct
  misc_feature 1..45: note = Flexizyme Fx
  source 1..45: mol_type = other RNA
ggatcgaaagatttccgcaggcccgaaagggtattggcgttaggt

SEQ ID NO: 2 - RNA, 45 nt, synthetic construct
  misc_feature 1..45: note = Flexizyme eFx
  source 1..45: mol_type = other RNA
ggatcgaaagatttccgcggccccgaaaggggattagcgttaggt

SEQ ID NO: 3 - RNA, 46 nt, synthetic construct
  misc_feature 1..46: note = Flexizyme dFx
  source 1..46: mol_type = other RNA
ggatcgaaagatttccgcatccccgaaagggtacatggcgttaggt

SEQ ID NO: 4 - RNA, 47 nt, synthetic construct
  misc_feature 1..47: note = Flexizyme aFx
  source 1..47: mol_type = other RNA
ggatcgaaagatttccgcacccccgaaaggggtaagtggcgttaggt